European Patent Specification EP 3 716 957 B1, published July 19, 2023. Title: Steroidal compounds for treatment of mental and neurological disorders. Applicant: Ustav organicke chemie a biochemie AV CR, v.v.i. et al. The sequence listing filed with the application follows.

SEQUENCE LISTING (20 sequences)

SEQ ID NO: 1 - protein, 34 aa, Homo sapiens
STLDSFMQPFQSTLWLLVGLSVHVVAVMLYLLDR

SEQ ID NO: 2 - protein, 34 aa, Homo sapiens
VSPSAFLEPFSASVWVMMFVMLLIVSAIAVFVFE

SEQ ID NO: 3 - protein, 34 aa, Homo sapiens
VSPSAFLEPFSADVWVMMFVMLLIVSAVAVFVFE

SEQ ID NO: 4 - protein, 34 aa, Homo sapiens
VSPSAFLEPYSPAVWVMMFVMCLTVVAITVFMFE

SEQ ID NO: 5 - protein, 34 aa, Homo sapiens
VSPSAFLEPYSPAVWVMMFVMCLTVVAVTVFIFE

SEQ ID NO: 6 - protein, 21 aa, Homo sapiens
SSAMWFSWGVLLNSGIGEGAP

SEQ ID NO: 7 - protein, 21 aa, Homo sapiens
GKAIWLLWGLVFNNSVPVQNP

SEQ ID NO: 8 - protein, 21 aa, Homo sapiens
GKAIWLLWGLVFNNSVPVQNP

SEQ ID NO: 9 - protein, 21 aa, Homo sapiens
GKSVWLLWALVFNNSVPIENP

SEQ ID NO: 10 - protein, 21 aa, Homo sapiens
GKSIWLLWALVFNNSVPVENP

SEQ ID NO: 11 - protein, 36 aa, Homo sapiens
RSFSARILGMVWAGFAMIIVASYTANLAAFLVLDRP

SEQ ID NO: 12 - protein, 36 aa, Homo sapiens
KGTTSKIMVSVWAFFAVIFLASYTANLAAFMIQEEF

SEQ ID NO: 13 - protein, 36 aa, Homo sapiens
KGTTSKIMVSVWAFFAVIFLASYTANLAAFMIQEEY

SEQ ID NO: 14 - protein, 36 aa, Homo sapiens
RGTTSKIMVLVWAFFAVIFLASYTANLAAFMIQEQY

SEQ ID NO: 15 - protein, 36 aa, Homo sapiens
RGTTSKIMVLVWAFFAVIFLASYTANLAAFMIQEEY

SEQ ID NO: 16 - protein, 31 aa, Homo sapiens
LTFENMAGVFMLVAGGIVAGIFLIFIEIAYK

SEQ ID NO: 17 - protein, 32 aa, Homo sapiens
LDIDNMAGVFYMLAAAMALSLITFIWEHLFYW

SEQ ID NO: 18 - protein, 32 aa, Homo sapiens
LDIDNMAGVFYMLGAAMALSLITFICEHLFYW

SEQ ID NO: 19 - protein, 32 aa, Homo sapiens
LDIDNMAGVFYMLLVAMGLALLVFAWEHLVYW

SEQ ID NO: 20 - protein, 32 aa, Homo sapiens
LDIDNMAGVFYMLLVAMGLSLLVFAWEHLVYW